European Patent Application EP 4 483 886 A1, published January 1, 2025. Title: RNA COMPOUNDS FOR TREATING PROLIFERATIVE DISORDERS. Applicant: Johann-Wolfgang-Goethe-Universität Frankfurt am Main. The sequence listing filed with the application follows.

SEQUENCE LISTING (3 sequences)

SEQ ID NO: 1 - protein, 393 aa, Homo sapiens [sequence omitted]

SEQ ID NO: 2 - protein, 416 aa, synthetic construct
MDYKDHDGDYKDHDIDYKDDDDKMEEPQSDPSVEPPLSQETFSDLWKLLPENNVLSPLPSQAMDDLMLSPDDIEQWFTEDPGPDEAPRMPEAAPPVAPAPAAPTPAAPAPAPSWPLSSSVPSQKTYQGSYGFRLGFLHSGTAKSVTCTYSPALNKMFCQLAKTCPVQLWVDSTPPPGTRVRAMAIYKQSQHMTEVVRRCPHHERCSDSDGLAPPQHLIRVEGNLRVEYLDDRNTFRHSVVVPYEPPEVGSDCTTIHYNYMCNSSCMGGMNRRPILTIITLEDSSGNLLGRNSFEVRVCACPGRDRRTEEENLRKKGEPHHELPPGSTKRALPNNTSSSPQPKKKPLDGEYFTLQIRGRERFEMFRELNEALELKDAQAGKEPGGSRAHSSHLKSKKGQSTSRHKKLMFKTEGPDSD

SEQ ID NO: 3 - RNA, 1249 nt, synthetic construct
  source 1..1249: mol_type = other RNA
atggactacaaagaccatgacggtgabataaagatcatgatatcgabacaaggatgacgatgacaagatggaggagccgcagtcagatcctagcgtcgagccccctctgagtcaggaaacattttcagacctatggaaactacttcctgaaaacaacgttctgtcccccttgccgtcccaagcaatggatgatttgatgctgtccccggacgatattgaacaatggttcactgaagacccaggtccagatgaagctcccagaatgccagaggctgctccccccgtggcccctgcaccagcagctcctacaccggcggcccctgcaccagccccctcctggcccctgtcatcttctgtcccttcccagaaaacctaccagggcagctacggtttccgtctgggcttcttgcattctgggacagccaagtctgtgacttgcacgtactcccctgccctcaacaagatgttttgccaactggccaagacctgccctgtgcagctgtgggttgattccacacccccgcccggcacccgcgtccgcgccatggccatctacaagcagtcacagcacatgacggaggttgtgaggcgctgcccccaccatgagcgctgctcagatagcgatggtctggcccctcctcagcatcttatccgagtggaaggaaatttgcgtgtggagtatttggatgacagaaacacttttcgacatagtgtggtggtgccctatgagccgcctgaggttggctctgactgtaccaccatccactacaactacatgtgtaacagttcctgcatgggcggcatgaaccggaggcccatcctcaccatcatcacactggaagactccagtggtaatctactgggacggaacagctttgaggtgcgtgtttgtgcctgtcctgggagagaccggcgcacagaggaagagaatctccgcaagaaaggggagcctcaccacgagctgcccccagggagcactaagcgagcactgcccaacaacaccagctcctctccccagccaaagaagaaaccactggatggagaatatttcacccttcagatccgtgggcgtgagcgcttcgagatgttccgagagctgaatgaggccttggaactcaaggatgcccaggctgggaaggagccaggggggagcagggctcactccagccacctgaagtccaaaaagggtcagtctacctcccgccataaaaaactcatgttcaagacagaagggcctgactcagactga